European Patent Application EP 4 279 090 A1, published November 22, 2023. Title: COMPOSITION. Applicant: ADC Therapeutics SA Medimmune Limited. The sequence listing filed with the application follows.

SEQUENCE LISTING (21 sequences)

SEQ ID NO: 1 - protein, 122 aa, Mus musculus
QVQLVESGGGVVQPGRSLRLSCAASGFTFSSYGMSWVRQAPGKGLEWVATISSGGSYTYYPDSVKGRFTISRDNSKNTLYLQMNSLRAEDTAVYYCARHPIYYTYDDTMDYWGQGTTVTVSS

SEQ ID NO: 2 - protein, 108 aa, Mus musculus
EIVLTQSPGTLSLSPGERATLSCSASSSVSSGNFHWYQQKPGLAPRLLIYRTSNLASGIPARFSGSGSGTDFTLTISSLEPEDFAVYYCQQWSGYPWTFGGGTKLEIK

SEQ ID NO: 3 - protein, 451 aa, Mus musculus
QVQLVESGGGVVQPGRSLRLSCAASGFTFSSYGMSWVRQAPGKGLEWVATISSGGSYTYYPDSVKGRFTISRDNSKNTLYLQMNSLRAEDTAVYYCARHPIYYTYDDTMDYWGQGTTVTVSSASTKGPSVFPLAPSSKSTSGGTAALGCLVKDYFPEPVTVSWNSGALTSGVHTFPAVLQSSGLYSLSSVVTVPSSSLGTQTYICNVNHKPSNTKVDKKVEPKSCDKTHTCPPCPAPELLGGPSVFLFPPKPKDTLMISRTPEVTCVVVDVSHEDPEVKFNWYVDGVEVHNAKTKPREEQYNSTYRVVSVLTVLHQDWLNGKEYKCKVSNKALPAPIEKTISKAKGQPREPQVYTLPPSREEMTKNQVSLTCLVKGFYPSDIAVEWESNGQPENNYKTTPPVLDSDGSFFLYSKLTVDKSRWQQGNVFSCSVMHEALHNHYTQKSLSLSPG

SEQ ID NO: 4 - protein, 215 aa, Mus musculus
EIVLTQSPGTLSLSPGERATLSCSASSSVSSGNFHWYQQKPGLAPRLLIYRTSNLASGIPARFSGSGSGTDFTLTISSLEPEDFAVYYCQQWSGYPWTFGGGTKLEIKRTVAAPSVFIFPPSDEQLKSGTASVVCLLNNFYPREAKVQWKVDNALQSGNSQESVTEQDSKDSTYSLSSTLTLSKADYEKHKVYACEVTHQGLSSPVTKSFNRGEC

SEQ ID NO: 5 - protein, 5 aa, Mus musculus
SYGMS

SEQ ID NO: 6 - protein, 17 aa, Mus musculus
TISSGGSYTYYPDSVKG

SEQ ID NO: 7 - protein, 13 aa, Mus musculus
HPIYYTYDDTMDY

SEQ ID NO: 8 - protein, 12 aa, Mus musculus
SASSSVSSGNFH

SEQ ID NO: 9 - protein, 7 aa, Mus musculus
RTSNLAS

SEQ ID NO: 10 - protein, 9 aa, Mus musculus
QQWSGYPWT

SEQ ID NO: 11 - protein, 121 aa, Mus musculus
QVQLVQSGAEVKKPGASVKVSCKGSGYTFTDYAMHWVRQAPGQGLEWIGVISTYYGNTNYNQKFKGKATMTVDKSTSTAYMELRSLRSDDTAVYYCARGGLREYYYAMDYWGQGTMVTVSS

SEQ ID NO: 12 - protein, 113 aa, Mus musculus
DIVMTQSPDSLAVSLGERATINCKSSQSLLNSSNQKNYLAWYQQKPGQPPKLLVYFASTRESGVPDRFSGSGSGTDFTLTISSLQAEDVAVYYCQQHYSTPPTFGQGTKLEIK

SEQ ID NO: 13 - protein, 450 aa, Mus musculus
QVQLVQSGAEVKKPGASVKVSCKGSGYTFTDYAMHWVRQAPGQGLEWIGVISTYYGNTNYNQKFKGKATMTVDKSTSTAYMELRSLRSDDTAVYYCARGGLREYYYAMDYWGQGTMVTVSSASTKGPSVFPLAPSSKSTSGGTAALGCLVKDYFPEPVTVSWNSGALTSGVHTFPAVLQSSGLYSLSSVVTVPSSSLGTQTYICNVNHKPSNTKVDKKVEPKSCDKTHTCPPCPAPELLGGPSVFLFPPKPKDTLMISRTPEVTCVVVDVSHEDPEVKFNWYVDGVEVHNAKTKPREEQYNSTYRVVSVLTVLHQDWLNGKEYKCKVSNKALPAPIEKTISKAKGQPREPQVYTLPPSREEMTKNQVSLTCLVKGFYPSDIAVEWESNGQPENNYKTTPPVLDSDGSFFLYSKLTVDKSRWQQGNVFSCSVMHEALHNHYTQKSLSLSPG

SEQ ID NO: 14 - protein, 220 aa, Mus musculus
DIVMTQSPDSLAVSLGERATINCKSSQSLLNSSNQKNYLAWYQQKPGQPPKLLVYFASTRESGVPDRFSGSGSGTDFTLTISSLQAEDVAVYYCQQHYSTPPTFGQGTKLEIKRTVAAPSVFIFPPSDEQLKSGTASVVCLLNNFYPREAKVQWKVDNALQSGNSQESVTEQDSKDSTYSLSSTLTLSKADYEKHKVYACEVTHQGLSSPVTKSFNRGEC

SEQ ID NO: 15 - protein, 5 aa, Mus musculus
DYAMH

SEQ ID NO: 16 - protein, 17 aa, Mus musculus
VISTYYGNTNYNQKFKG

SEQ ID NO: 17 - protein, 12 aa, Mus musculus
GGLREYYYAMDY

SEQ ID NO: 18 - protein, 17 aa, Mus musculus
KSSQSLLNSSNQKNYLA

SEQ ID NO: 19 - protein, 7 aa, Mus musculus
FASTRES

SEQ ID NO: 20 - protein, 9 aa, Mus musculus
QQHYSTPPT

SEQ ID NO: 21 - protein, 451 aa, Mus musculus
QVQLVQSGAEVKKPGASVKVSCKGSGYTFTDYAMHWVRQAPGQGLEWIGVISTYYGNTNYNQKFKGKATMTVDKSTSTAYMELRSLRSDDTAVYYCARGGLREYYYAMDYWGQGTMVTVSSASTKGPSVFPLAPSSKSTSGGTAALGCLVKDYFPEPVTVSWNSGALTSGVHTFPAVLQSSGLYSLSSVVTVPSSSLGTQTYICNVNHKPSNTKVDKKVEPKSCDKTHTCPPCPAPELLGGPSVFLFPPKPKDTLMISRTPEVTCVVVDVSHEDPEVKFNWYVDGVEVHNAKTKPREEQYNSTYRVVSVLTVLHQDWLNGKEYKCKVSNKALPAPIEKTISKAKGQPREPQVYTLPPSREEMTKNQVSLTCLVKGFYPSDIAVEWESNGQPENNYKTTPPVLDSDGSFFLYSKLTVDKSRWQQGNVFSCSVMHEALHNHYTQKSLSLSPGK